European Patent Application EP 4 180 450 A1, published May 17, 2023. Title: PEPTIDES AND COMBINATION OF PEPTIDES FOR USE IN IMMUNOTHERAPY AGAINST NON-SMALL CELL LUNG CANCER AND OTHER CANCERS. Applicant: immatics biotechnologies GmbH. The sequence listing filed with the application follows.

SEQUENCE LISTING (25 sequences)

SEQ ID NO: 1 - protein, 9 aa, Homo sapiens
KVLEHVVRV

SEQ ID NO: 2 - protein, 9 aa, Homo sapiens
KVLEHVVRL

SEQ ID NO: 3 - protein, 9 aa, Homo sapiens
KVLEHVVRA

SEQ ID NO: 4 - protein, 9 aa, Homo sapiens
KVLEHVVRI

SEQ ID NO: 5 - protein, 9 aa, Homo sapiens
KLLEHVVRV

SEQ ID NO: 6 - protein, 9 aa, Homo sapiens
KLLEHVVRL

SEQ ID NO: 7 - protein, 9 aa, Homo sapiens
KLLEHVVRA

SEQ ID NO: 8 - protein, 9 aa, Homo sapiens
KLLEHVVRI

SEQ ID NO: 9 - protein, 9 aa, Homo sapiens
KALEHVVRV

SEQ ID NO: 10 - protein, 9 aa, Homo sapiens
KALEHVVRL

SEQ ID NO: 11 - protein, 9 aa, Homo sapiens
KALEHVVRA

SEQ ID NO: 12 - protein, 9 aa, Homo sapiens
KALEHVVRI

SEQ ID NO: 13 - protein, 9 aa, Homo sapiens
YLLEHVVRV

SEQ ID NO: 14 - protein, 9 aa, Homo sapiens
YLLEHVVRL

SEQ ID NO: 15 - protein, 9 aa, Homo sapiens
YLLEHVVRA

SEQ ID NO: 16 - protein, 9 aa, Homo sapiens
YLLEHVVRI

SEQ ID NO: 17 - protein, 9 aa, Homo sapiens
YALEHVVRV

SEQ ID NO: 18 - protein, 9 aa, Homo sapiens
YALEHVVRL

SEQ ID NO: 19 - protein, 9 aa, Homo sapiens
YALEHVVRA

SEQ ID NO: 20 - protein, 9 aa, Homo sapiens
YALEHVVRI

SEQ ID NO: 21 - protein, 9 aa, Homo sapiens
YVLEHVVRV

SEQ ID NO: 22 - protein, 9 aa, Homo sapiens
YVLEHVVRL

SEQ ID NO: 23 - protein, 9 aa, Homo sapiens
YVLEHVVRA

SEQ ID NO: 24 - protein, 9 aa, Homo sapiens
YVLEHVVRI

SEQ ID NO: 25 - protein, 9 aa, Homo sapiens
  SITE 1: note = misc_feature - Xaa can be Lys or Tyr
  SITE 2: note = misc_feature - Xaa can be Val, Leu or Ala
  SITE 9: note = misc_feature - Xaa can be Val, Leu, Ala or Ile
XXLEHVVRX